European Patent Specification EP 3 757 228 B1, published April 17, 2024. Title: Multiplex Detection of Nucleic Acids. Applicant: Dahl, Carl OF Ericsson, John O. The sequence listing filed with the application follows.

SEQUENCE LISTING (3 sequences)

SEQ ID NO: 1 - DNA, 93 bp, Artificial Sequence
  Synthetic oligonucleotide
  misc_feature (31)..(60): positions 31 to 60 represent a target complementary sequence on human chromosome 21.
atgtgacccttccgtctgttgagttaggccnnnnnnnnnnnnnnnnnnnnnnnnnnnnnntcgtgccttgtcattcgggagcactaactgctg

SEQ ID NO: 2 - DNA, 152 bp, Artificial Sequence
  Synthetic oligonucleotide
  misc_feature (1)..(1): c has 5' phosphate
  misc_feature (64)..(73): n is a, c, g, or t
cgcacacgattaaggtccagtcacaggcagagatcggaagagcgtcgtgtagggaaagagtgtnnnnnnnnnngtgtagatctcggtggtcgccgtatcatttcatgctgctaacggtcgagtcggacaggtggctccactaaatagacgca

SEQ ID NO: 3 - DNA, 152 bp, Artificial Sequence
  Synthetic oligonucleotide
  misc_feature (1)..(1): g has a 5' phosphate
  misc_feature (64)..(73): n is a, c, g, or t
ggcctaactcaacagacggaagggtcacatagatcggaagagcgtcgtgtagggaaagagtgtnnnnnnnnnngtgtagatctcggtggtcgccgtatcatttcatgctgctaacggtcgagcagttagtgctcccgaatgacaaggcacga